European Patent Application EP 4 600 261 A1, published August 13, 2025. Title: keratin YK93-2, AND preparation method thereof, pharmaceutical composition thereof and use thereof. Applicant: Institute of Materia Medica Chinese Academy Of Medical Sciences. The sequence listing filed with the application follows.

SEQUENCE LISTING (2 sequences)

SEQ ID NO: 1 - protein, 502 aa, Manis pentadactyla
MTCGSGFCGRTFSCASACGPRPGRCCITAAPYSGVSCYRGITGAFGSRSVCGAFRSGSCGRSFGYRAGGVCGPSPPCITSVSVNESLLTPLNLEIDPSAQCVKQEEKEQIKSLNSRFAAFIDKVRFLEQQNKLLETKWQFYQNRQCCESNLEPLFQGYIETLRREAECAEADSGRLASELNHVQEVLEGYKKKYEEEVALRATAENEFVALKKDVDCAYLRKSDLEANAEALIQEIDFLRRLYEEEIRVLQSHISDTSVIVKMDNSRDLNMDCIVAEIKAQYDDIASRSRAEAESWYRTKCEEIKATVIRHGETLRRTKEEINELNRMIQRLTAEVENAKCQNSKLEAAVAQAEQQGEAALNDARCKLAGLEAALQKAKQDMACLLKEYQEVMNSKLGLDIEIATYRRLLEGEEQRLCEGIGAVNVCVSSSRGGVVCGDLTVSGTRPVTGSNCSAPCSGNLAVSTGICAPCGPCNSITSCGLGSYGISSYGVGSCASSCRKC

SEQ ID NO: 2 - DNA, 1506 bp, Manis pentadactyla
  source 1..1506: mol_type = genomic DNA
atgacctgtggtagcggcttttgtggtcgtacctttagctgcgcaagcgcatgcggcccgcgccctggtagatgttgcattaccgcagccccgtatagtggtgtgagctgttatcgcggcattaccggcgcatttggcagtcgcagtgtgtgcggcgcctttcgtagtggcagctgcggccgtagttttggttatcgcgcaggtggtgtgtgcggtccgagtccgccgtgtattaccagtgttagcgtgaatgaaagcctgctgaccccgctgaatctggaaattgatccgagtgcccagtgcgtgaaacaggaagaaaaagaacagattaagagtctgaatagccgttttgcagcattcattgataaagtgcgttttctggaacagcagaataagctgctggaaaccaaatggcagttttatcagaatcgccagtgttgcgaaagcaatctggaaccgctgtttcagggttatattgaaaccctgcgtcgcgaagccgaatgcgccgaagcagatagtggtcgtctggccagcgaactgaatcatgtgcaggaagtgctggaaggctataaaaagaaatatgaagaagaggttgccctgcgtgcaaccgcagaaaatgaatttgtggccctgaaaaaagatgtggattgtgcatatctgcgcaaaagtgatctggaagcaaatgcagaagccctgattcaggaaattgattttctgcgtcgtctgtatgaagaagaaattcgcgtgctgcagagccatattagcgataccagtgtgattgttaaaatggataatagtcgtgatctgaatatggattgcattgtggcagaaattaaggcacagtatgatgatattgcaagccgtagccgcgccgaagccgaaagttggtatcgcaccaaatgcgaagaaattaaggccaccgtgattcgtcatggcgaaaccctgcgccgtaccaaagaagaaattaatgaactgaatcgcatgattcagcgtctgaccgccgaagtggaaaatgcaaaatgccagaatagtaaactggaagcagcagttgcacaggccgaacagcagggtgaagcagccctgaatgatgcccgttgtaaactggcaggcctggaagcagccttacagaaagcaaaacaggatatggcatgcctgctgaaagaatatcaggaagttatgaatagcaagctgggcctggatattgaaattgccacctatcgccgtctgctggaaggcgaagaacagcgtctgtgtgaaggcattggcgccgttaatgtttgtgtgagtagcagccgcggcggtgtggtgtgcggcgatctgaccgttagcggtacccgtccggttaccggtagtaattgtagcgcaccgtgcagcggtaatctggccgtgagtaccggcatttgtgccccgtgcggcccgtgtaatagcattaccagctgtggcctgggtagctatggcattagtagttatggtgttggtagttgcgcaagcagttgtcgcaaatgt